European Patent Specification EP 3 294 774 B1, published August 28, 2024. Title: AFUCOSYLATED PROTEIN, CELL AND METHODS THEREOF. Applicant: ZUMUTOR BIOLOGICS, INC. Application 194/CHE/2015. The sequence listing filed with the application follows.

SEQUENCE LISTING (28 sequences)

SEQ ID NO: 1 - DNA, 3126 bp, Cricetulus griseus
  Cricetulus griseus Fut8 mRNA (1)..(3126)
caggttgctgctctggcttaggccatctatgaccctggtggtgttttcattcactataagtccttcccatctttattaactgagcaagttcagctagtaattttagagaccgaggttcaagcaataacacctatctctgcaataccgtgtggctttcttcaatgtcttacatcctaaggaaaggaagcatgtagagcccaggaagcacaggacaagaaagctgcctccttgtatcaccaggaagatctttttgtaagagtcatcacagtataccagagagactaattttgtctgaagcatcatgtgttgaaacaacagaaacttattttcctgtgtggctaactagaaccagagtacaatgtttccaattctttgagctccgagaagacagaagggagttgaaactctgaaaatgcgggcatggactggttcctggcgttggattatgctcattctttttgcctgggggaccttattgttttatataggtggtcatttggttcgagataatgaccaccctgaccattctagcagagaactctccaagattcttgcaaagctggagcgcttaaaacaacaaaatgaagacttgaggagaatggctgagtctctccgaataccagaaggccctattgatcaggggacagctacaggaagagtccgtgttttagaagaacagcttgttaaggccaaagaacagattgaaaattacaagaaacaagctaggaatgatctgggaaaggatcatgaaatcttaaggaggaggattgaaaatggagctaaagagctctggttttttctacaaagtgaattgaagaaattaaagaaattagaaggaaacgaactccaaagacatgcagatgaaattcttttggatttaggacatcatgaaaggtctatcatgacagatctatactacctcagtcaaacagatggagcaggtgagtggcgggaaaaagaagccaaagatctgacagagctggtccagcggagaataacatatctgcagaatcccaaggactgcagcaaagccagaaagctggtatgtaatatcaacaaaggctgtggctatggatgtcaactccatcatgtggtttactgcttcatgattgcttatggcacccagcgaacactcatcttggaatctcagaattggcgctatgctactggaggatgggagactgtgtttagacctgtaagtgagacatgcacagacaggtctggcctctccactggacactggtcaggtgaagtgaaggacaaaaatgttcaagtggtcgagctccccattgtagacagcctccatcctcgtcctccttacttacccttggctgtaccagaagaccttgcagatcgactcctgagagtccatggtgatcctgcagtgtggtgggtatcccagtttgtcaaatacttgatccgtccacaaccttggctggaaagggaaatagaagaaaccaccaagaagcttggcttcaaacatccagttattggagtccatgtcagacgcactgacaaagtgggaacagaagcagccttccatcccattgaggaatacatggtacacgttgaagaacattttcagcttctcgaacgcagaatgaaagtggataaaaaaagagtgtatctggccactgatgacccttctttgttaaaggaggcaaagacaaagtactccaattatgaatttattagtgataactctatttcttggtcagctggactacacaaccgatacacagaaaattcacttcggggcgtgatcctggatatacactttctctcccaggctgacttccttgtgtgtactttttcatcccaggtctgtagggttgcttatgaaatcatgcaaacactgcatcctgatgcctctgcaaacttccattctttagatgacatctactattttggaggccaaaatgcccacaaccagattgcagtttatcctcaccaacctcgaactaaagaggaaatccccatggaacctggagatatcattggtgtggctggaaaccattggaatggttactctaaaggtgtcaacagaaaactaggaaaaacaggcctgtacccttcctacaaagtccgagagaagatagaaacagtcaaataccctacatatcctgaagctgaaaaatagagatggagtgtaagagattaacaacagaatttagttcagaccatctcagccaagcagaagacccagactaacatatggttcattgacagacatgctccgcaccaagagcaagtgggaaccctcagatgctgcactggtggaacgcctctttgtgaagggctgctgtgccctcaagcccatgcacagtaaaataatgtactcacacataacatacaaatggattattttctactttgccctttaaatattctgtccccatgaaacaaacactgccacattatgtaatttaagtgacacagacgttttgtgtgagacttcaaacatggtgcctatatctgagagacctctgtgatttactgagaagatgagaacagctcccttctgtggggaagttggttcttagtcagtggtggactggccactgaattcactgcaatcaacagattcagaatgagaatggatgtttttcctttatatggttgtctggattttttttaaagtaatttcatcagttcagttcatccacctcattaataaatgaaggaatataccaataaaatcaaatgaaatattcactgtccattaggaagttttataaaacaatgccatgaacaaaaaattctttagtactcaatgtttctggacattctctttgataacaaaaataaattttaaaaaggaattttgtaaagtttctgggattctgtatcactggatgatgtagttataagctttgtagtagaaatatgggaagtgggtttatagcttttaagatttttttctacttttgtcctactttttctatttctgatagaataatcatatttcaagagaagcattggtcccctctaatactagtaactgcctttagtcatgcatattatatgaagttgctaagaacacgctttgggggaggtgttcactctcttagtttgatattgttgacttgatataattgaatgaaatagtcattctcttgcttccag

SEQ ID NO: 2 - DNA, 4101 bp, Streptococcus pyogenes
  Cas9 nucleotide sequence (1)..(4101)
gacaagaagtacagcatcggcctggccatcggcaccaactctgtgggctgggccgtgatcaccgacgagtacaaggtgcccagcaagaaattcaaggtgctgggcaacaccgaccggcacagcatcaagaagaacctgatcggagccctgctgttcgacagcggcgaaacagccgaggccacccggctgaagagaaccgccagaagaagatacaccagacggaagaaccggatctgctatctgcaagagatcttcagcaacgagatggccaaggtggacgacagcttcttccacagactggaagagtccttcctggtggaagaggataagaagcacgagcggcaccccatcttcggcaacatcgtggacgaggtggcctaccacgagaagtaccccaccatctaccacctgagaaagaaactggtggacagcaccgacaaggccgacctgcggctgatctatctggccctggcccacatgatcaagttccggggccacttcctgatcgagggcgacctgaaccccgacaacagcgacgtggacaagctgttcatccagctggtgcagacctacaaccagctgttcgaggaaaaccccatcaacgccagcggcgtggacgccaaggccatcctgtctgccagactgagcaagagcagacggctggaaaatctgatcgcccagctgcccggcgagaagaagaatggcctgttcggaaacctgattgccctgagcctgggcctgacccccaacttcaagagcaacttcgacctggccgaggatgccaaactgcagctgagcaaggacacctacgacgacgacctggacaacctgctggcccagatcggcgaccagtacgccgacctgtttctggccgccaagaacctgtccgacgccatcctgctgagcgacatcctgagagtgaacaccgagatcaccaaggcccccctgagcgcctctatgatcaagagatacgacgagcaccaccaggacctgaccctgctgaaagctctcgtgcggcagcagctgcctgagaagtacaaagagattttcttcgaccagagcaagaacggctacgccggctacattgacggcggagccagccaggaagagttctacaagttcatcaagcccatcctggaaaagatggacggcaccgaggaactgctcgtgaagctgaacagagaggacctgctgcggaagcagcggaccttcgacaacggcagcatcccccaccagatccacctgggagagctgcacgccattctgcggcggcaggaagatttttacccattcctgaaggacaaccgggaaaagatcgagaagatcctgaccttccgcatcccctactacgtgggccctctggccaggggaaacagcagattcgcctggatgaccagaaagagcgaggaaaccatcaccccctggaacttcgaggaagtggtggacaagggcgcttccgcccagagcttcatcgagcggatgaccaacttcgataagaacctgcccaacgagaaggtgctgcccaagcacagcctgctgtacgagtacttcaccgtgtataacgagctgaccaaagtgaaatacgtgaccgagggaatgagaaagcccgccttcctgagcggcgagcagaaaaaggccatcgtggacctgctgttcaagaccaaccggaaagtgaccgtgaagcagctgaaagaggactacttcaagaaaatcgagtgcttcgactccgtggaaatctccggcgtggaagatcggttcaacgcctccctgggcacataccacgatctgctgaaaattatcaaggacaaggacttcctggacaatgaggaaaacgaggacattctggaagatatcgtgctgaccctgacactgtttgaggacagagagatgatcgaggaacggctgaaaacctatgcccacctgttcgacgacaaagtgatgaagcagctgaagcggcggagatacaccggctggggcaggctgagccggaagctgatcaacggcatccgggacaagcagtccggcaagacaatcctggatttcctgaagtccgacggcttcgccaacagaaacttcatgcagctgatccacgacgacagcctgacctttaaagaggacatccagaaagcccaggtgtccggccagggcgatagcctgcacgagcacattgccaatctggccggcagccccgccattaagaagggcatcctgcagacagtgaaggtggtggacgagctcgtgaaagtgatgggccggcacaagcccgagaacatcgtgatcgaaatggccagagagaaccagaccacccagaagggacagaagaacagccgcgagagaatgaagcggatcgaagagggcatcaaagagctgggcagccagatcctgaaagaacaccccgtggaaaacacccagctgcagaacgagaagctgtacctgtactacctgcagaatgggcgggatatgtacgtggaccaggaactggacatcaaccggctgtccgactacgatgtggaccatatcgtgcctcagagctttctgaaggacgactccatcgacaacaaggtgctgaccagaagcgacaagaaccggggcaagagcgacaacgtgccctccgaagaggtcgtgaagaagatgaagaactactggcggcagctgctgaacgccaagctgattacccagagaaagttcgacaatctgaccaaggccgagagaggcggcctgagcgaactggataaggccggcttcatcaagagacagctggtggaaacccggcagatcacaaagcacgtggcacagatcctggactcccggatgaacactaagtacgacgagaatgacaagctgatccgggaagtgaaagtgatcaccctgaagtccaagctggtgtccgatttccggaaggatttccagttttacaaagtgcgcgagatcaacaactaccaccacgcccacgacgcctacctgaacgccgtcgtgggaaccgccctgatcaaaaagtaccctaagctggaaagcgagttcgtgtacggcgactacaaggtgtacgacgtgcggaagatgatcgccaagagcgagcaggaaatcggcaaggctaccgccaagtacttcttctacagcaacatcatgaactttttcaagaccgagattaccctggccaacggcgagatccggaagcggcctctgatcgagacaaacggcgaaaccggggagatcgtgtgggataagggccgggattttgccaccgtgcggaaagtgctgagcatgccccaagtgaatatcgtgaaaaagaccgaggtgcagacaggcggcttcagcaaagagtctatcctgcccaagaggaacagcgataagctgatcgccagaaagaaggactgggaccctaagaagtacggcggcttcgacagccccaccgtggcctattctgtgctggtggtggccaaagtggaaaagggcaagtccaagaaactgaagagtgtgaaagagctgctggggatcaccatcatggaaagaagcagcttcgagaagaatcccatcgactttctggaagccaagggctacaaagaagtgaaaaaggacctgatcatcaagctgcctaagtactccctgttcgagctggaaaacggccggaagagaatgctggcctctgccggcgaactgcagaagggaaacgaactggccctgccctccaaatatgtgaacttcctgtacctggccagccactatgagaagctgaagggctcccccgaggataatgagcagaaacagctgtttgtggaacagcacaagcactacctggacgagatcatcgagcagatcagcgagttctccaagagagtgatcctggccgacgctaatctggacaaagtgctgtccgcctacaacaagcaccgggataagcccatcagagagcaggccgagaatatcatccacctgtttaccctgaccaatctgggagcccctgccgccttcaagtactttgacaccaccatcgaccggaagaggtacaccagcaccaaagaggtgctggacgccaccctgatccaccagagcatcaccggcctgtacgagacacggatcgacctgtctcagctgggaggcgac

SEQ ID NO: 3 - DNA, 4101 bp, Streptococcus pyogenes; identical to SEQ ID NO: 2
  Cas9n nucleotide sequence (1)..(4101)

SEQ ID NO: 4 - DNA, 238 bp, Cricetulus griseus
  Fut8 Exon 7 nucleotide sequence (1)..(238)
aatcccaaggactgcagcaaagccagaaagctggtatgtaatatcaacaaaggctgtggctatggatgtcaactccatcatgtggtttactgcttcatgattgcttatggcacccagcgaacactcatcttggaatctcagaattggcgctatgctactggaggatgggagactgtgtttagacctgtaagtgagacatgcacagacaggtctggcctctccactggacactggtcag

SEQ ID NO: 5 - protein, 79 aa, Cricetulus griseus
  Fut8 Exon 7 amino acid sequence (1)..(79)
NPKDCSKARKLVCNINKGCGYGCQLHHVVYCFMIAYGTQRTLILESQNWRYATGGWETVFRPVSETCTDRSGLSTGHWS

SEQ ID NO: 6 - DNA, 23 bp, Artificial Sequence
  CRISPR recognition sequence 1
aattggcgctatgctactggagg

SEQ ID NO: 7 - RNA, 23 nt, Artificial Sequence
  gRNA1
aauuggcgcuaugcuacuggagg

SEQ ID NO: 8 - DNA, 23 bp, Artificial Sequence
  CRISPR recognition sequence 2
ccagcgaacactcatcttggaat

SEQ ID NO: 9 - RNA, 23 nt, Artificial Sequence
  gRNA2
ccagcgaacacucaucuuggaau

SEQ ID NO: 10 - DNA, 499 bp, Artificial Sequence
  gRNA + scaffold for Fut8 Exon 7
  misc_feature (1)..(499)
attccaagatgagtgttcgcgttttagagctagaaatagcaagttaaaataaggctagtccgttatcaacttgaaaaagtggcaccgagtcggtgcttttttgctccgcggcacgagaactcaaagccccggggcctgggtcccacgcggggtcccttacccagggtgccccgggcgctcatttgcatgtcccacccaacaggtaaacctgacaggtcatcgcggccaggtacgacctggcggtcagagcaccaaacatacgagccttgtgatgagttccgttgcatgaaattctcccaaaggctccaagatggacaggaaagggcgcggttcggtcaccgtaagtagaataggtgaaagactcccgtgccttataaggcctgtgggtgacttcttctcaccgaattggcgctatgctactgggttttagagctagaaatagcaagttaaaataaggctagtccgttatcaacttgaaaaagtggcaccgagtcggtgc

SEQ ID NO: 11 - DNA, 20 bp, Artificial Sequence
  CRISPR DNA binding domain 1
attccaagatgagtgttcgc

SEQ ID NO: 12 - RNA, 20 nt, Artificial Sequence
  Target specific crRNA sequence
auuccaagaugaguguucgc

SEQ ID NO: 13 - DNA, 20 bp, Artificial Sequence
  DNA Binding domain 2
aattggcgctatgctactgg

SEQ ID NO: 14 - RNA, 20 nt, Artificial Sequence
  Target specific crRNA sequence
aauuggcgcuaugcuacugg

SEQ ID NO: 15 - DNA, 76 bp, Artificial Sequence
  gRNA scaffold
gttttagagctagaaatagcaagttaaaataaggctagtccgttatcaacttgaaaaagtggcaccgagtcggtgc

SEQ ID NO: 16 - protein, 469 aa, Artificial Sequence
  Anti-her2 antibody heavy chain amino acid sequence
MGWSCIILFLVATATGVHSEVQLVESGGGLVQPGGSLRLSCAASGFNIKDTYIHWVRQAPGKGLEWVARIYPTNGYTRYADSVKGRFTISADTSKNTAYLQMNSLRAEDTAVYYCSRWGGDGFYAMDYWGQGTLVTVSSASTKGPSVFPLAPSSKSTSGGTAALGCLVKDYFPEPVTVSWNSGALTSGVHTFPAVLQSSGLYSLSSVVTVPSSSLGTQTYICNVNHKPSNTKVDKKVEPKSCDKTHTCPPCPAPELLGGPSVFLFPPKPKDTLMISRTPEVTCVVVDVSHEDPEVKFNWYVDGVEVHNAKTKPREEQYNSTYRVVSVLTVLHQDWLNGKEYKCKVSNKALPAPIEKTISKAKGQPREPQVYTLPPSREEMTKNQVSLTCLVKGFYPSDIAVEWESNGQPENNYKTTPPVLDSDGSFFLYSKLTVDKSRWQQGNVFSCSVMHEALHNHYTQKSLSLSPGK

SEQ ID NO: 17 - protein, 233 aa, Artificial Sequence
  Antiher2 antibody light chain amino acid sequence
MGWSCIILFLVATATGVHSDIQMTQSPSSLSASVGDRVTITCRASQDVNTAVAWYQQKPGKAPKLLIYSASFLYSGVPSRFSGSRSGTDFTLTISSLQPEDFATYYCQQHYTTPPTFGQGTKVEIKRTVAAPSVFIFPPSDEQLKSGTASVVCLLNNFYPREAKVQWKVDNALQSGNSQESVTEQDSKDSTYSLSSTLTLSKADYEKHKVYACEVTHQGLSSPVTKSFNRGEC

SEQ ID NO: 18 - DNA, 26 bp, Artificial Sequence
  FORWARD PRIMER
aagaaataagctgaatcagctctgac

SEQ ID NO: 19 - DNA, 23 bp, Artificial Sequence
  REVERSE PRIMER
gtgctaatctgacctaaccagag

SEQ ID NO: 20 - DNA, 394 bp, Cricetulus griseus
  Fut8 Exon 7 and associated intron sequences (1)..(394)
aagaaataagctgaatcagctctgacttattgtgtgattttcaatacctgtgaccaaaatgagaagttaactccttatatctttatcttatttgtttctctggaagaatcccaaggactgcagcaaagccagaaagctggtatgtaatatcaacaaaggctgtggctatggatgtcaactccatcatgtggtttactgcttcatgattgcttatggcacccagcgaacactcatcttggaatctcagaattggcgctatgctactggaggatgggagactgtgtttagacctgtaagtgagacatgcacagacaggtctggcctctccactggacactggtcaggtaaggagcatgtgcaccatgaaagatctctggttaggtcagattagcac

SEQ ID NO: 21 - DNA, 189 bp, Cricetulus griseus
  Clone CR2TMCHO 1A allelic version (1)..(189)
aatcccaaggactgcagcaaagccagaaagctggtatgtaatatcaacaaaggctgtggctatggatgtcaactccatcatgtggtttactgcttcatgattgcttatggcacccagcgaacactctgtttagacctgtaagtgagacatgcacagacaggtctggcctctccactggacactggtcag

SEQ ID NO: 22 - DNA, 697 bp, Cricetulus griseus
  Clone CR2TMCHO 1A allelic version (1)..(697)
aatcccaaggactgcagcaaagccagaaagctggtatgtaatatcaacaaaggctgtggctatggatgtcaactccatcatgtggtttactgcttcatgactcacggggatttccaagtctccaccccattgacgtcaatgggagtttgttttggcaccaaaatcaacgggactttccaaaatgtcgtaataaccccgccccgttgacgcaaatgggcggtaggcgtgtacggtgggaggtctatataagcagagctcgtttagtgaaccgtcagatcactagaagctttattgcggtagtttatcacagttaaattgctaacgcagtcaggccaacagagaccacacccaagctggccgccaccatggccccaaagaagaagcggaaggtcggtatccacggagtcccagcagccgacaagaagtacagcatcggcctggccatcggcaccaactctgtgggctgggccgtgatcaccgacgagtacaaggtgcccagcaagaaattcaaggtgctgggcaacaccgaccggcacagcatcaagaagaacctgatcggagccctgctgttcgacagcggcgaaacagccgaggccacccggctgaagagaaccgccagaaggatgggagactgtgtttagacctgtaagtgagacatgcacagacaggtctggcctctccactggacactggtcag

SEQ ID NO: 23 - DNA, 417 bp, Cricetulus griseus
  Clone CR2TMCHO 1B allelic version (1)..(417)
aatcccaaggactgcagcaaagccagaaagctggtatgtaatatcaacaaaggctgtggctatggatgtcaactccatcatgtggtttactgcttcatgattgcttatggcacccagcgaacactcatctggaggatgggagactgtgtttagacctgtaagtgagacatgcacagacaggtctggcctctccactggacactggtcaaatcccaaggactgcagcaaagccagaaagctggtatgtaatatcaacaaaggctgtggctatggatgtcaactccatcatgtggtttactgcttcatgattgcttatggcacccagcgaacactcatctggaggatgggagactgtgtttagacctgtaagtgagacatgcacagacaggtctggcctctccactggacactggtcag

SEQ ID NO: 24 - DNA, 378 bp, Cricetulus griseus
  Clone CR2TMCHO 1B allelic version (1)..(378)
aatcccaaggactgcagcaaagccagaaagctggtatgtaatatcaacaaaggctgtggctatggatgtcaactccatcatgtggtttactgcttcatgattgcttatggcacccagttgcctaatagaacaacctttgcctggttgttacaaaatatattctctgtaccagtatctagttttacaatgagctatggaatgttaatgatttatttgtctacattataaattatattgctttgatttgctctaagtggaacaaacactcatcttggaatctcagaattggcgctatgctactggaggatgggagactgtgtttagacctgtaagtgagacatgcacagacaggtctggcctctccactggacactggtc

SEQ ID NO: 25 - protein, 46 aa, Cricetulus griseus
  Frame shift with STOP CODON (1)..(46Frame shift with STOP CODON)
NPKDCSKARKLVCNINKGCGYGCQLHHVVYCFMIAYGTQRTLCLDL

SEQ ID NO: 26 - protein, 68 aa, Cricetulus griseus
  Frame shift with STOP CODON (1)..(68)
NPKDCSKARKLVCNINKGCGYGCQLHHVVYCFMTHGDFQVSTPLTSMGVCFGTKINGTFQNVVITPPR

SEQ ID NO: 27 - protein, 50 aa, Cricetulus griseus
  Frame shift with STOP CODON (1)..(50)
NPKDCSKARKLVCNINKGCGYGCQLHHVVYCFMIAYGTQRTLIWRMGDCV

SEQ ID NO: 28 - protein, 75 aa, Cricetulus griseus
  Frame shift with STOP CODON (1)..(75)
NPKDCSKARKLVCNINKGCGYGCQLHHVVYCFMIAYGTQLPNRTTFAWLLQNIFSVPVSSFTMSYGMLMIYLSTL